European Patent Application EP 4 585 683 A1, published July 16, 2025. Title: 一种用于预防乙型肝炎病毒感染的药物组合物及其应用. Applicant: 远大赛威信生命科学（南京）有限公司. The sequence listing filed with the application follows.

SEQUENCE LISTING (4 sequences)

SEQ ID NO: 1 - protein, 226 aa, synthetic construct
MENITSGFLGPLLVLQAGFFLLTRILTIPQSLDSWWTSLNFLGGSPVCLGQNSQSPTSNHSPTSCPPICPGYRWMCLRRFIIFLFILLLCLIFLLVLLDYQGMLPVCPLIPGSTTTSTGPCKTCTTPAQGNSMFPSCCCTKPTDGNCTCIPIPSSWAFAKYLWEWASVRFSWLSLLVPFVQWFVGLSPTVWLSAIWMMWYWGPSLYSIVSPFIPLLPIFFCLWVYI

SEQ ID NO: 2 - DNA, 21 bp, synthetic construct
  source 1..21: mol_type = other DNA
tcgttcgttcgttcgttcgtt

SEQ ID NO: 3 - DNA, 25 bp, synthetic construct
  source 1..25: mol_type = other DNA
tcgttcgttcgttcgttcgttcgtt

SEQ ID NO: 4 - DNA, 21 bp, synthetic construct
  source 1..21: mol_type = other DNA
tcgtcgtcgtcgtcgtcgtcg